European Patent Application EP 4 681 773 A2, published January 21, 2026. Title: Novel Compound and Application Thereof. Applicant: KYLONOVA (XIAMEN) BIOPHARMA CO., LTD. The sequence listing filed with the application follows.

SEQUENCE LISTING (92 sequences)

SEQ ID NO: 1 - RNA, 19 nt, synthetic construct
  source 1..19: mol_type = other RNA
gggtttttcttgttgacaa

SEQ ID NO: 2 - RNA, 19 nt, synthetic construct
  source 1..19: mol_type = other RNA
ttgtcaacaagaaaaaccc

SEQ ID NO: 3 - RNA, 19 nt, synthetic construct
  source 1..19: mol_type = other RNA
ggtttttcttgttgacaaa

SEQ ID NO: 4 - RNA, 19 nt, synthetic construct
  source 1..19: mol_type = other RNA
tttgtcaacaagaaaaacc

SEQ ID NO: 5 - RNA, 19 nt, synthetic construct
  source 1..19: mol_type = other RNA
gtttttcttgttgacaaaa

SEQ ID NO: 6 - RNA, 19 nt, synthetic construct
  source 1..19: mol_type = other RNA
ttttgtcaacaagaaaaac

SEQ ID NO: 7 - RNA, 19 nt, synthetic construct
  source 1..19: mol_type = other RNA
gaccgtgtgcacttcgctt

SEQ ID NO: 8 - RNA, 19 nt, synthetic construct
  source 1..19: mol_type = other RNA
aagcgaagtgcacacggtc

SEQ ID NO: 9 - RNA, 19 nt, synthetic construct
  source 1..19: mol_type = other RNA
accgtgtgcacttcgcttc

SEQ ID NO: 10 - RNA, 19 nt, synthetic construct
  source 1..19: mol_type = other RNA
gaagcgaagtgcacacggt

SEQ ID NO: 11 - RNA, 19 nt, synthetic construct
  source 1..19: mol_type = other RNA
ccgtgtgcacttcgcttca

SEQ ID NO: 12 - RNA, 19 nt, synthetic construct
  source 1..19: mol_type = other RNA
tgaagcgaagtgcacacgg

SEQ ID NO: 13 - RNA, 19 nt, synthetic construct
  source 1..19: mol_type = other RNA
cgtgtgcacttcgcttcac

SEQ ID NO: 14 - RNA, 19 nt, synthetic construct
  source 1..19: mol_type = other RNA
gtgaagcgaagtgcacacg

SEQ ID NO: 15 - RNA, 19 nt, synthetic construct
  source 1..19: mol_type = other RNA
gtgtgcacttcgcttcacc

SEQ ID NO: 16 - RNA, 19 nt, synthetic construct
  source 1..19: mol_type = other RNA
ggtgaagcgaagtgcacac

SEQ ID NO: 17 - RNA, 19 nt, synthetic construct
  source 1..19: mol_type = other RNA
tgtgcacttcgcttcacct

SEQ ID NO: 18 - RNA, 19 nt, synthetic construct
  source 1..19: mol_type = other RNA
aggtgaagcgaagtgcaca

SEQ ID NO: 19 - RNA, 19 nt, synthetic construct
  source 1..19: mol_type = other RNA
cagcaatgtcaacgaccga

SEQ ID NO: 20 - RNA, 19 nt, synthetic construct
  source 1..19: mol_type = other RNA
ggtcgttgacattgctgaa

SEQ ID NO: 21 - RNA, 19 nt, synthetic construct
  source 1..19: mol_type = other RNA
ggatgtgtctgcggcgttt

SEQ ID NO: 22 - RNA, 19 nt, synthetic construct
  source 1..19: mol_type = other RNA
aaacgccgcagacacatcc

SEQ ID NO: 23 - RNA, 19 nt, synthetic construct
  source 1..19: mol_type = other RNA
tggatgtgtctgcggcgtt

SEQ ID NO: 24 - RNA, 19 nt, synthetic construct
  source 1..19: mol_type = other RNA
aacgccgcagacacatcca

SEQ ID NO: 25 - RNA, 19 nt, synthetic construct
  source 1..19: mol_type = other RNA
ctggatgtgtctgcggcgt

SEQ ID NO: 26 - RNA, 19 nt, synthetic construct
  source 1..19: mol_type = other RNA
acgccgcagacacatccag

SEQ ID NO: 27 - RNA, 19 nt, synthetic construct
  source 1..19: mol_type = other RNA
cggggcgcacctctcttta

SEQ ID NO: 28 - RNA, 19 nt, synthetic construct
  source 1..19: mol_type = other RNA
taaagagaggtgcgccccg

SEQ ID NO: 29 - RNA, 19 nt, synthetic construct
  source 1..19: mol_type = other RNA
ggggcgcacctctctttac

SEQ ID NO: 30 - RNA, 19 nt, synthetic construct
  source 1..19: mol_type = other RNA
gtaaagagaggtgcgcccc

SEQ ID NO: 31 - RNA, 19 nt, synthetic construct
  source 1..19: mol_type = other RNA
ggcgcacctctctttacgc

SEQ ID NO: 32 - RNA, 19 nt, synthetic construct
  source 1..19: mol_type = other RNA
gcgtaaagagaggtgcgcc

SEQ ID NO: 33 - RNA, 19 nt, synthetic construct
  source 1..19: mol_type = other RNA
gcgcacctctctttacgcg

SEQ ID NO: 34 - RNA, 19 nt, synthetic construct
  source 1..19: mol_type = other RNA
cgcgtaaagagaggtgcgc

SEQ ID NO: 35 - RNA, 19 nt, synthetic construct
  source 1..19: mol_type = other RNA
tcttgttggttcttctgga

SEQ ID NO: 36 - RNA, 19 nt, synthetic construct
  source 1..19: mol_type = other RNA
tccagaagaaccaacaaga

SEQ ID NO: 37 - RNA, 19 nt, synthetic construct
  source 1..19: mol_type = other RNA
ttcttgttggttcttctgg

SEQ ID NO: 38 - RNA, 19 nt, synthetic construct
  source 1..19: mol_type = other RNA
ccagaagaaccaacaagaa

SEQ ID NO: 39 - RNA, 19 nt, synthetic construct
  source 1..19: mol_type = other RNA
cttgttggttcttctggac

SEQ ID NO: 40 - RNA, 19 nt, synthetic construct
  source 1..19: mol_type = other RNA
gtccagaagaaccaacaag

SEQ ID NO: 41 - RNA, 19 nt, synthetic construct
  source 1..19: mol_type = other RNA
ttgttggttcttctggact

SEQ ID NO: 42 - RNA, 19 nt, synthetic construct
  source 1..19: mol_type = other RNA
agtccagaagaaccaacaa

SEQ ID NO: 43 - RNA, 21 nt, synthetic construct
  source 1..21: mol_type = other RNA
  misc_feature 1..21: note = the first and second nucleotides from the 3' end of the sense strand are 2'-deoxythymidine, 2' -OH of the nucleotides at positions 7, 9, 10, 11 from the 5' end of the sense strand is replaced by fluorine, 2' -OH of the remaining nucleotides in the sense strand is replaced by methoxy group, and there are two consecutive phosphorothioate linkages between 3 adjacent nucleotides at the 5' and 3' ends of the sense strand
gggtttttcttgttgacaatt

SEQ ID NO: 44 - RNA, 21 nt, synthetic construct
  source 1..21: mol_type = other RNA
  misc_feature 1..21: note = 2' -OH of the nucleotides at positions 2, 6, 8, 9, 10, 14, 15, 16 from the 5' end of the antisense strand is replaced by fluorine, 2' -OH of the remaining nucleotides in the antisense strand is replaced by methoxy group, and there are two consecutive phosphorothioate linkages between 3 adjacent nucleotides at the 5' and 3' ends of the antisense strand
ttgtcaacaagaaaaaccctt

SEQ ID NO: 45 - RNA, 21 nt, synthetic construct
  source 1..21: mol_type = other RNA
  misc_feature 1..21: note = 2' -OH of the nucleotides at positions 7, 9, 10, 11 from the 5' end of the sense strand is replaced by fluorine, 2' -OH of the remaining nucleotides in the sense strand is replaced by methoxy group, and there are two consecutive phosphorothioate linkages between 3 adjacent nucleotides at the 5' and 3' ends of the sense strand
gggtttttcttgttgacaatt

SEQ ID NO: 46 - RNA, 21 nt, synthetic construct
  source 1..21: mol_type = other RNA
  misc_feature 1..21: note = 2' -OH of the nucleotides at positions 2, 5, 7, 8, 9, 13, 14, 15 from the 5' end of the antisense strand is replaced by fluorine, 2' -OH of the remaining nucleotides in the antisense strand is replaced by methoxy group, and there are two consecutive phosphorothioate linkages between 3 adjacent nucleotides at the 5' and 3' ends of the antisense strand
ttgtcaacaagaaaaacccat

SEQ ID NO: 47 - RNA, 21 nt, synthetic construct
  source 1..21: mol_type = other RNA
  misc_feature 1..21: note = 2' -OH of the nucleotides at positions 7, 9, 10, 11 from the 5' end of the sense strand is replaced by fluorine, 2' -OH of the remaining nucleotides in the sense strand is replaced by methoxy group, and there are two consecutive phosphorothioate linkages between 3 adjacent nucleotides at the 5' and 3' ends of the sense strand
ggtttttcttgttgacaaaat

SEQ ID NO: 48 - RNA, 21 nt, synthetic construct
  source 1..21: mol_type = other RNA
  misc_feature 1..21: note = 2' -OH of the nucleotides at positions 2, 6, 7, 8, 12, 13, 14, 15 from the 5' end of the antisense strand is replaced by fluorine, 2' -OH of the remaining nucleotides in the antisense strand is replaced by methoxy group, and there are two consecutive phosphorothioate linkages between 3 adjacent nucleotides at the 5' and 3' ends of the antisense strand
tttgtcaacaagaaaaacctt

SEQ ID NO: 49 - RNA, 21 nt, synthetic construct
  source 1..21: mol_type = other RNA
  misc_feature 1..21: note = 2' -OH of the nucleotides at positions 7, 9, 10, 11 from the 5' end of the sense strand is replaced by fluorine, 2' -OH of the remaining nucleotides in the sense strand is replaced by methoxy group, and there are two consecutive phosphorothioate linkages between 3 adjacent nucleotides at the 5' and 3' ends of the sense strand
gtttttcttgttgacaaaatt

SEQ ID NO: 50 - RNA, 21 nt, synthetic construct
  source 1..21: mol_type = other RNA
  misc_feature 1..21: note = 2' -OH of the nucleotides at positions 2, 6, 8, 9, 10, 14, 15, 16 from the 5' end of the antisense strand is replaced by fluorine, 2' -OH of the remaining nucleotides in the antisense strand is replaced by methoxy group, and there are two consecutive phosphorothioate linkages between 3 adjacent nucleotides at the 5' and 3' ends of the antisense strand
ttttgtcaacaagaaaaactt

SEQ ID NO: 51 - RNA, 21 nt, synthetic construct
  source 1..21: mol_type = other RNA
  misc_feature 1..21: note = 2' -OH of the nucleotides at positions 2, 4, 9, 10, 11 from the 5' end of the sense strand is replaced by fluorine, 2' -OH of the remaining nucleotides in the sense strand is replaced by methoxy group, and there are two consecutive phosphorothioate linkages between 3 adjacent nucleotides at the 5' and 3' ends of the sense strand
gaccgtgtgcacttcgcttat

SEQ ID NO: 52 - RNA, 21 nt, synthetic construct
  source 1..21: mol_type = other RNA
  misc_feature 1..21: note = the first and second nucleotides from the 3' end of the antisense strand are 2'-deoxythymidine, 2' -OH of the nucleotides at positions 2, 6, 8, 9, 10, 14, 15, 16 from the 5' end of the antisense strand is replaced by fluorine, 2' -OH of the remaining nucleotides in the antisense strand is replaced by methoxy group, and there are two consecutive phosphorothioate linkages between 3 adjacent nucleotides at the 5' and 3' ends of the antisense strand
aagcgaagtgcacacggtctt

SEQ ID NO: 53 - RNA, 21 nt, synthetic construct
  source 1..21: mol_type = other RNA
  misc_feature 1..21: note = the first and second nucleotides from the 3' end of the sense strand are 2' -deoxythymidine, 2' -OH of the nucleotides at positions 6, 8, 9, 10 from the 5' end of the sense strand is replaced by fluorine, 2' -OH of the remaining nucleotides in the sense strand is replaced by methoxy group, and there are two consecutive phosphorothioate linkages between 3 adjacent nucleotides at the 5' and 3' ends of the sense strand
accgtgtgcacttcgcttctt

SEQ ID NO: 54 - RNA, 21 nt, synthetic construct
  source 1..21: mol_type = other RNA
  misc_feature 1..21: note = 2' -OH of the nucleotides at positions 2, 6, 8, 9, 10, 14, 15, 16 from the 5' end of the antisense strand is replaced by fluorine, 2' -OH of the remaining nucleotides in the antisense strand is replaced by methoxy group, and there are two consecutive phosphorothioate linkages between 3 adjacent nucleotides at the 5' and 3' ends of the antisense strand
gaagcgaagtgcacacggttt

SEQ ID NO: 55 - RNA, 21 nt, synthetic construct
  source 1..21: mol_type = other RNA
  misc_feature 1..21: note = 2' -OH of the nucleotides at positions 2, 4, 6, 8, 10, 15 from the 5' end of the sense strand is replaced by fluorine, 2' -OH of the remaining nucleotides in the sense strand is replaced by methoxy group, and there are two consecutive phosphorothioate linkages between 3 adjacent nucleotides at the 5' and 3' ends of the sense strand
accgtgtgcacttcgcttcat

SEQ ID NO: 56 - RNA, 21 nt, synthetic construct
  source 1..21: mol_type = other RNA
  misc_feature 1..21: note = the first and second nucleotides from the 3' end of the antisense strand are 2' -deoxythymidine, 2' -OH of the nucleotides at positions 2, 6, 8, 9, 10, 14, 15, 16 from the 5' end of the antisense strand is replaced by fluorine, 2' -OH of the remaining nucleotides in the antisense strand is replaced by methoxy group, and there are two consecutive phosphorothioate linkages between 3 adjacent nucleotides at the 5' and 3' ends of the antisense strand
gaagcgaagtgcacacggttt

SEQ ID NO: 57 - RNA, 21 nt, synthetic construct
  source 1..21: mol_type = other RNA
  misc_feature 1..21: note = the first and second nucleotides from the 3' end of the sense strand are 2' -deoxythymidine, 2' -OH of the nucleotides at positions 7, 9, 10, 11 from the 5' end of the sense strand is replaced by fluorine, 2' -OH of the remaining nucleotides in the sense strand is replaced by methoxy group, and there are two consecutive phosphorothioate linkages between 3 adjacent nucleotides at the 5' and 3' ends of the sense strand
ccgtgtgcacttcgcttcatt

SEQ ID NO: 58 - RNA, 21 nt, synthetic construct
  source 1..21: mol_type = other RNA
  misc_feature 1..21: note = 2' -OH of the nucleotides at positions 2, 6, 8, 9, 10, 14, 15, 16 from the 5' end of the antisense strand is replaced by fluorine, 2' -OH of the remaining nucleotides in the antisense strand is replaced by methoxy group, and there are two consecutive phosphorothioate linkages between 3 adjacent nucleotides at the 5' and 3' ends of the antisense strand
tgaagcgaagtgcacacggtt

SEQ ID NO: 59 - RNA, 21 nt, synthetic construct
  source 1..21: mol_type = other RNA
  misc_feature 1..21: note = 2' -OH of the nucleotides at positions 7, 9, 10, 11 from the 5' end of the sense strand is replaced by fluorine, 2' -OH of the remaining nucleotides in the sense strand is replaced by methoxy group, and there are two consecutive phosphorothioate linkages between 3 adjacent nucleotides at the 5' and 3' ends of the sense strand
cgtgtgcacttcgcttcactt

SEQ ID NO: 60 - RNA, 21 nt, synthetic construct
  source 1..21: mol_type = other RNA
  misc_feature 1..21: note = 2' -OH of the nucleotides at positions 2, 6, 8, 9, 10, 14, 15, 16 from the 5' end of the antisense strand is replaced by fluorine, 2' -OH of the remaining nucleotides in the antisense strand is replaced by methoxy group, and there are two consecutive phosphorothioate linkages between 3 adjacent nucleotides at the 5' and 3' ends of the antisense strand
gtgaagcgaagtgcacacgtt

SEQ ID NO: 61 - RNA, 21 nt, synthetic construct
  source 1..21: mol_type = other RNA
  misc_feature 1..21: note = 2' -OH of the nucleotides at positions 6, 8, 9, 10 from the 5' end of the sense strand is replaced by fluorine, 2' -OH of the remaining nucleotides in the sense strand is replaced by methoxy group, and there are two consecutive phosphorothioate linkages between 3 adjacent nucleotides at the 5' and 3' ends of the sense strand
gtgtgcacttcgcttcaccat

SEQ ID NO: 62 - RNA, 21 nt, synthetic construct
  source 1..21: mol_type = other RNA
  misc_feature 1..21: note = 2' -OH of the nucleotides at positions 2, 6, 8, 9, 10, 14, 15, 16 from the 5' end of the antisense strand is replaced by fluorine, 2' -OH of the remaining nucleotides in the antisense strand is replaced by methoxy group, and there are two consecutive phosphorothioate linkages between 3 adjacent nucleotides at the 5' and 3' ends of the antisense strand
ggtgaagcgaagtgcacacat

SEQ ID NO: 63 - RNA, 21 nt, synthetic construct
  source 1..21: mol_type = other RNA
  misc_feature 1..21: note = 2' -OH of the nucleotides at positions 7, 9, 10, 11, 12 from the 5' end of the sense strand is replaced by fluorine, 2' -OH of the remaining nucleotides in the sense strand is replaced by methoxy group, and there are two consecutive phosphorothioate linkages between 3 adjacent nucleotides at the 5' and 3' ends of the sense strand
tgtgcacttcgcttcacctat

SEQ ID NO: 64 - RNA, 21 nt, synthetic construct
  source 1..21: mol_type = other RNA
  misc_feature 1..21: note = 2' -OH of the nucleotides at positions 2, 6, 8, 9, 10, 14, 15, 16 from the 5' end of the antisense strand is replaced by fluorine, 2' -OH of the remaining nucleotides in the antisense strand is replaced by methoxy group, and there are two consecutive phosphorothioate linkages between 3 adjacent nucleotides at the 5' and 3' ends of the antisense strand
aggtgaagcgaagtgcacaat

SEQ ID NO: 65 - RNA, 21 nt, synthetic construct
  source 1..21: mol_type = other RNA
  misc_feature 1..21: note = 2' -OH of the nucleotides at positions 7, 9, 10, 11 from the 5' end of the sense strand is replaced by fluorine, 2' -OH of the remaining nucleotides in the sense strand is replaced by methoxy group, and there are two consecutive phosphorothioate linkages between 3 adjacent nucleotides at the 5' and 3' ends of the sense strand
cagcaatgtcaacgaccgaat

SEQ ID NO: 66 - RNA, 21 nt, synthetic construct
  source 1..21: mol_type = other RNA
  misc_feature 1..21: note = 2' -OH of the nucleotides at positions 2, 6, 8, 9, 10, 14, 15, 16 from the 5' end of the antisense strand is replaced by fluorine, 2' -OH of the remaining nucleotides in the antisense strand is replaced by methoxy group, and there are two consecutive phosphorothioate linkages between 3 adjacent nucleotides at the 5' and 3' ends of the antisense strand
ggtcgttgacattgctgaaat

SEQ ID NO: 67 - RNA, 21 nt, synthetic construct
  source 1..21: mol_type = other RNA
  misc_feature 1..21: note = 2' -OH of the nucleotides at positions 7, 9, 10, 11 from the 5' end of the sense strand is replaced by fluorine, 2' -OH of the remaining nucleotides in the sense strand is replaced by methoxy group, and there are two consecutive phosphorothioate linkages between 3 adjacent nucleotides at the 5' and 3' ends of the sense strand
ggatgtgtctgcggcgtttat

SEQ ID NO: 68 - RNA, 21 nt, synthetic construct
  source 1..21: mol_type = other RNA
  misc_feature 1..21: note = the first and second nucleotides from the 3' end of the antisense strand are 2' -deoxythymidine, 2' -OH of the nucleotides at positions 2, 6, 8, 9, 10, 14, 15, 16 from the 5' end of the antisense strand is replaced by fluorine, 2' -OH of the remaining nucleotides in the antisense strand is replaced by methoxy group, and there are two consecutive phosphorothioate linkages between 3 adjacent nucleotides at the 5' and 3' ends of the antisense strand
aaacgccgcagacacatcctt

SEQ ID NO: 69 - RNA, 21 nt, synthetic construct
  source 1..21: mol_type = other RNA
  misc_feature 1..21: note = 2' -OH of the nucleotides at positions 7, 9, 10, 11 from the 5' end of the sense strand is replaced by fluorine, 2' -OH of the remaining nucleotides in the sense strand is replaced by methoxy group, and there are two consecutive phosphorothioate linkages between 3 adjacent nucleotides at the 5' and 3' ends of the sense strand
tggatgtgtctgcggcgttat

SEQ ID NO: 70 - RNA, 21 nt, synthetic construct
  source 1..21: mol_type = other RNA
  misc_feature 1..21: note = the first and second nucleotides from the 3' end of the antisense strand are 2' -deoxythymidine, 2' -OH of the nucleotides at positions 2, 6, 8, 9, 10, 14, 15, 16 from the 5' end of the antisense strand is replaced by fluorine, 2' -OH of the remaining nucleotides in the antisense strand is replaced by methoxy group, and there are two consecutive phosphorothioate linkages between 3 adjacent nucleotides at the 5' and 3' ends of the antisense strand
aacgccgcagacacatccatt

SEQ ID NO: 71 - RNA, 21 nt, synthetic construct
  source 1..21: mol_type = other RNA
  misc_feature 1..21: note = 2' -OH of the nucleotides at positions 7, 9, 10, 11 from the 5' end of the sense strand is replaced by fluorine, 2' -OH of the remaining nucleotides in the sense strand is replaced by methoxy group, and there are two consecutive phosphorothioate linkages between 3 adjacent nucleotides at the 5' and 3' ends of the sense strand
ctggatgtgtctgcggcgtta

SEQ ID NO: 72 - RNA, 21 nt, synthetic construct
  source 1..21: mol_type = other RNA
  misc_feature 1..21: note = the first and second nucleotides from the 3' end of the antisense strand are 2' -deoxythymidine, 2' -OH of the nucleotides at positions 2, 6, 8, 9, 10, 14, 15, 16 from the 5' end of the antisense strand is replaced by fluorine, 2' -OH of the remaining nucleotides in the antisense strand is replaced by methoxy group, and there are two consecutive phosphorothioate linkages between 3 adjacent nucleotides at the 5' and 3' ends of the antisense strand
acgccgcagacacatccagtt

SEQ ID NO: 73 - RNA, 21 nt, synthetic construct
  source 1..21: mol_type = other RNA
  misc_feature 1..21: note = 2' -OH of the nucleotides at positions 7, 9, 10, 11 from the 5' end of the sense strand is replaced by fluorine, 2' -OH of the remaining nucleotides in the sense strand is replaced by methoxy group, and there are two consecutive phosphorothioate linkages between 3 adjacent nucleotides at the 5' and 3' ends of the sense strand
cggggcgcacctctctttata

SEQ ID NO: 74 - RNA, 21 nt, synthetic construct
  source 1..21: mol_type = other RNA
  misc_feature 1..21: note = 2' -OH of the nucleotides at positions 2, 6, 8, 9, 10, 14, 15, 16 from the 5' end of the antisense strand is replaced by fluorine, 2' -OH of the remaining nucleotides in the antisense strand is replaced by methoxy group, and there are two consecutive phosphorothioate linkages between 3 adjacent nucleotides at the 5' and 3' ends of the antisense strand
taaagagaggtgcgccccgtt

SEQ ID NO: 75 - RNA, 21 nt, synthetic construct
  source 1..21: mol_type = other RNA
  misc_feature 1..21: note = 2' -OH of the nucleotides at positions 2, 4, 6, 8, 10, 12, 14, 16, 18 from the 5' end of the sense strand is replaced by fluorine, 2' -OH of the remaining nucleotides in the sense strand is replaced by methoxy group, and there are two consecutive phosphorothioate linkages between 3 adjacent nucleotides at the 5' and 3' ends of the sense strand
cggggcgcacctctctttatt

SEQ ID NO: 76 - RNA, 21 nt, synthetic construct
  source 1..21: mol_type = other RNA
  misc_feature 1..21: note = the first and second nucleotides from the 3' end of the antisense strand are 2' -deoxythymidine, 2' -OH of the nucleotides at positions 2, 6, 8, 9, 10, 14, 15, 16 from the 5' end of the antisense strand is replaced by fluorine, 2' -OH of the remaining nucleotides in the antisense strand is replaced by methoxy group, and there are two consecutive phosphorothioate linkages between 3 adjacent nucleotides at the 5' and 3' ends of the antisense strand
taaagagaggtgcgccccgtt

SEQ ID NO: 77 - RNA, 21 nt, synthetic construct
  source 1..21: mol_type = other RNA
  misc_feature 1..21: note = 2' -OH of the nucleotides at positions 7, 9, 10, 11 from the 5' end of the sense strand is replaced by fluorine, 2' -OH of the remaining nucleotides in the sense strand is replaced by methoxy group, and there are two consecutive phosphorothioate linkages between 3 adjacent nucleotides at the 5' and 3' ends of the sense strand
ggggcgcacctctctttacta

SEQ ID NO: 78 - RNA, 21 nt, synthetic construct
  source 1..21: mol_type = other RNA
  misc_feature 1..21: note = the first and second nucleotides from the 3' end of the antisense strand are 2' -deoxythymidine, 2' -OH of the nucleotides at positions 2, 5, 7, 8, 10, 14, 15, 16 from the 5' end of the antisense strand is replaced by fluorine, 2' -OH of the remaining nucleotides in the antisense strand is replaced by methoxy group, and there are two consecutive phosphorothioate linkages between 3 adjacent nucleotides at the 5' and 3' ends of the antisense strand
gtaaagagaggtgcgcccctt

SEQ ID NO: 79 - RNA, 21 nt, synthetic construct
  source 1..21: mol_type = other RNA
  misc_feature 1..21: note = 2' -OH of the nucleotides at positions 7, 9, 10, 11 from the 5' end of the sense strand is replaced by fluorine, 2' -OH of the remaining nucleotides in the sense strand is replaced by methoxy group, and there are two consecutive phosphorothioate linkages between 3 adjacent nucleotides at the 5' and 3' ends of the sense strand
ggcgcacctctctttacgcat

SEQ ID NO: 80 - RNA, 21 nt, synthetic construct
  source 1..21: mol_type = other RNA
  misc_feature 1..21: note = the first and second nucleotides from the 3' end of the antisense strand are 2' -deoxythymidine, 2' -OH of the nucleotides at positions 2, 6, 8, 9, 10, 14, 15, 16 from the 5' end of the antisense strand is replaced by fluorine, 2' -OH of the remaining nucleotides in the antisense strand is replaced by methoxy group, and there are two consecutive phosphorothioate linkages between 3 adjacent nucleotides at the 5' and 3' ends of the antisense strand
gcgtaaagagaggtgcgcctt

SEQ ID NO: 81 - RNA, 21 nt, synthetic construct
  source 1..21: mol_type = other RNA
  misc_feature 1..21: note = 2' -OH of the nucleotides at positions 7, 9, 10, 11 from the 5' end of the sense strand is replaced by fluorine, 2' -OH of the remaining nucleotides in the sense strand is replaced by methoxy group, and there are two consecutive phosphorothioate linkages between 3 adjacent nucleotides at the 5' and 3' ends of the sense strand
gcgcacctctctttacgcgta

SEQ ID NO: 82 - RNA, 21 nt, synthetic construct
  source 1..21: mol_type = other RNA
  misc_feature 1..21: note = the first and second nucleotides from the 3' end of the antisense strand are 2' -deoxythymidine, 2' -OH of the nucleotides at positions 2, 6, 8, 9, 10, 14, 15, 16 from the 5' end of the antisense strand is replaced by fluorine, 2' -OH of the remaining nucleotides in the antisense strand is replaced by methoxy group, and there are two consecutive phosphorothioate linkages between 3 adjacent nucleotides at the 5' and 3' ends of the antisense strand
cgcgtaaagagaggtgcgctt

SEQ ID NO: 83 - RNA, 21 nt, synthetic construct
  source 1..21: mol_type = other RNA
  misc_feature 1..21: note = 2' -OH of the nucleotides at positions 7, 9, 10, 11 from the 5' end of the sense strand is replaced by fluorine, 2' -OH of the remaining nucleotides in the sense strand is replaced by methoxy group, and there are two consecutive phosphorothioate linkages between 3 adjacent nucleotides at the 5' and 3' ends of the sense strand
tcttgttggttcttctggaat

SEQ ID NO: 84 - RNA, 21 nt, synthetic construct
  source 1..21: mol_type = other RNA
  misc_feature 1..21: note = 2' -OH of the nucleotides at positions 2, 6, 8, 9, 10, 14, 15, 16 from the 5' end of the antisense strand is replaced by fluorine, 2' -OH of the remaining nucleotides in the antisense strand is replaced by methoxy group, and there are two consecutive phosphorothioate linkages between 3 adjacent nucleotides at the 5' and 3' ends of the antisense strand
tccagaagaaccaacaagata

SEQ ID NO: 85 - RNA, 21 nt, synthetic construct
  source 1..21: mol_type = other RNA
  misc_feature 1..21: note = 2' -OH of the nucleotides at positions 3, 7, 9, 10, 11 from the 5' end of the sense strand is replaced by fluorine, 2' -OH of the remaining nucleotides in the sense strand is replaced by methoxy group, and there are two consecutive phosphorothioate linkages between 3 adjacent nucleotides at the 5' and 3' ends of the sense strand
tcttgttggttcttctggata

SEQ ID NO: 86 - RNA, 21 nt, synthetic construct
  source 1..21: mol_type = other RNA
  misc_feature 1..21: note = 2' -OH of the nucleotides at positions 2, 6, 8, 9, 10, 14, 15, 16 from the 5' end of the antisense strand is replaced by fluorine, 2' -OH of the remaining nucleotides in the antisense strand is replaced by methoxy group, and there are two consecutive phosphorothioate linkages between 3 adjacent nucleotides at the 5' and 3' ends of the antisense strand
tccagaagaaccaacaagaat

SEQ ID NO: 87 - RNA, 21 nt, synthetic construct
  source 1..21: mol_type = other RNA
  misc_feature 1..21: note = 2' -OH of the nucleotides at positions 6, 8, 9, 10 from the 5' end of the sense strand is replaced by fluorine, 2' -OH of the remaining nucleotides in the sense strand is replaced by methoxy group, and there are two consecutive phosphorothioate linkages between 3 adjacent nucleotides at the 5' and 3' ends of the sense strand
ttcttgttggttcttctggat

SEQ ID NO: 88 - RNA, 21 nt, synthetic construct
  source 1..21: mol_type = other RNA
  misc_feature 1..21: note = 2' -OH of the nucleotides at positions 2, 6, 8, 9, 10, 14, 15, 16 from the 5' end of the antisense strand is replaced by fluorine, 2' -OH of the remaining nucleotides in the antisense strand is replaced by methoxy group, and there are two consecutive phosphorothioate linkages between 3 adjacent nucleotides at the 5' and 3' ends of the antisense strand
ccagaagaaccaacaagaaat

SEQ ID NO: 89 - RNA, 21 nt, synthetic construct
  source 1..21: mol_type = other RNA
  misc_feature 1..21: note = 2' -OH of the nucleotides at positions 7, 9, 10, 11 from the 5' end of the sense strand is replaced by fluorine, 2' -OH of the remaining nucleotides in the sense strand is replaced by methoxy group, and there are two consecutive phosphorothioate linkages between 3 adjacent nucleotides at the 5' and 3' ends of the sense strand
cttgttggttcttctggacat

SEQ ID NO: 90 - RNA, 21 nt, synthetic construct
  source 1..21: mol_type = other RNA
  misc_feature 1..21: note = 2' -OH of the nucleotides at positions 2, 6, 8, 9, 10, 14, 15, 16 from the 5' end of the antisense strand is replaced by fluorine, 2' -OH of the remaining nucleotides in the antisense strand is replaced by methoxy group, and there are two consecutive phosphorothioate linkages between 3 adjacent nucleotides at the 5' and 3' ends of the antisense strand
gtccagaagaaccaacaagta

SEQ ID NO: 91 - RNA, 21 nt, synthetic construct
  source 1..21: mol_type = other RNA
  misc_feature 1..21: note = 2' -OH of the nucleotides at positions 6, 8, 9, 10 from the 5' end of the sense strand is replaced by fluorine, 2' -OH of the remaining nucleotides in the sense strand is replaced by methoxy group, and there are two consecutive phosphorothioate linkages between 3 adjacent nucleotides at the 5' and 3' ends of the sense strand
ttgttggttcttctggactat

SEQ ID NO: 92 - RNA, 21 nt, synthetic construct
  source 1..21: mol_type = other RNA
  misc_feature 1..21: note = 2' -OH of the nucleotides at positions 2, 6, 8, 9, 10, 14, 15, 16 from the 5' end of the antisense strand is replaced by fluorine, 2' -OH of the remaining nucleotides in the antisense strand is replaced by methoxy group, and there are two consecutive phosphorothioate linkages between 3 adjacent nucleotides at the 5' and 3' ends of the antisense strand
agtccagaagaaccaacaaat